European Patent Application EP 4 289 952 A1, published December 13, 2023. Title: CHEMICALLY MODIFIED SMALL ACTIVATING RNA. Applicant: Ractigen Therapeutics. Application EP22749093.5. The sequence listing filed with the application follows.

SEQUENCE LISTING (25 sequences)

SEQ ID NO: 1 - DNA, 21 bp, Artificial Sequence
  Primer sequence
atcaccatcttccaggagcga

SEQ ID NO: 2 - DNA, 21 bp, Artificial Sequence
  Primer sequence
ttctccatggtggtgaagacg

SEQ ID NO: 3 - DNA, 20 bp, Artificial Sequence
  Primer sequence
ggaagaccatgtggacctgt

SEQ ID NO: 4 - DNA, 20 bp, Artificial Sequence
  Primer sequence
ggattagggcttcctcttgg

SEQ ID NO: 5 - RNA, 19 nt, Artificial Sequence
  Chemically modified oligonucleotide
  modified_base (1)..(19): (1,2,18,19)=2'-O-methyl(2'-OMe)
ccaacucauucuccaaguc

SEQ ID NO: 6 - RNA, 21 nt, Artificial Sequence
  Chemically modified oligonucleotide
  modified_base (1)..(20): (1,3,4,5,12,16,17,20)=2'-fluoro
uacuuggagaaugaguuggca

SEQ ID NO: 7 - RNA, 21 nt, Artificial Sequence
  Chemically modified oligonucleotide
  modified_base (1)..(20): (1,5,12,17,20)=2'-fluoro
uacuuggagaaugaguuggca

SEQ ID NO: 8 - RNA, 21 nt, Artificial Sequence
  Chemically modified oligonucleotide
  modified_base (1)..(20): (1,3,4,5,12,16,17,20)=2'-fluoro
  modified_base (2)..(21): (2,6,7,8,9,10,11,13,14,15,18,19,21)=2'-O-methyl(2'-OMe)
uacuuggagaaugaguuggca

SEQ ID NO: 9 - RNA, 21 nt, Artificial Sequence
  Chemically modified oligonucleotide
  modified_base (1)..(20): (1,5,12,17,20)=2'-fluoro
  modified_base (19)..(21): (19,20,21)=phosphorothioate (PS) backbone modification
uacuuggagaaugaguuggca

SEQ ID NO: 10 - RNA, 21 nt, Artificial Sequence
  Chemically modified oligonucleotide
  modified_base (5)..(20): (5,12,17,20)=2'-fluoro
  modified_base (19)..(21): (19,20,21)=phosphorothioate (PS) backbone modification
uacuuggagaaugaguuggca

SEQ ID NO: 11 - RNA, 21 nt, Artificial Sequence
  Chemically modified oligonucleotide
  modified_base (1)..(21): (1,2,3,19,20,21)=phosphorothioate (PS) backbone modification
  modified_base (1)..(20): (1,3,4,5,12,16,17,20)=2'-fluoro
uacuuggagaaugaguuggca

SEQ ID NO: 12 - RNA, 21 nt, Artificial Sequence
  Chemically modified oligonucleotide
  modified_base (2)..(21): (2,3,19,20,21)=phosphorothioate (PS) backbone modification
  modified_base (3)..(20): (3,4,5,12,16,17,20)=2'-fluoro
uacuuggagaaugaguuggca

SEQ ID NO: 13 - DNA, 21 bp, Artificial Sequence
  Chemically modified oligonucleotide
  modified_base (1)..(17): (1,2,9,13,14,17)=2'-fluoro
  misc_feature (1)..(21): (1,5,6,7,8,9,10,11,12,13,14,15,1,61,7,18,19,20,21)=RNA
  misc_feature (2)..(4): (2,3,4)=DNA
  modified_base (16)..(18): (16,17,18)=phosphorothioate (PS) backbone modification
uactuggagaaugaguuggca

SEQ ID NO: 14 - RNA, 19 nt, Artificial Sequence
  Chemically modified oligonucleotide
  modified_base (1)..(19): (1,2,18,19)=2'-fluoro
ccaacucauucuccaaguc

SEQ ID NO: 15 - RNA, 19 nt, Artificial Sequence
  Chemically modified oligonucleotide
  modified_base (1)..(2): (1,2)=2'-O-methyl(2'-OMe)
  modified_base (17)..(19): (17,18,19)=phosphorothioate (PS) backbone modification
ccaacucauucuccaaguc

SEQ ID NO: 16 - RNA, 19 nt, Artificial Sequence
  Chemically modified oligonucleotide
  modified_base (1)..(2): (1,2)=2'-fluoro
  modified_base (17)..(19): (17,18,19)=phosphorothioate (PS) backbone modification
ccaacucauucuccaaguc

SEQ ID NO: 17 - RNA, 19 nt, Artificial Sequence
  Chemically modified oligonucleotide
ccaacucauucuccaaguc

SEQ ID NO: 18 - DNA, 21 bp, Artificial Sequence
  Chemically modified oligonucleotide
  misc_feature (1)..(21): (1,5,6,7,8,9,10,11,12,13,14,15,16,17,18,19,20,21)=RNA
  misc_feature (2)..(4): (2,3,4)=DNA
uactuggagaaugaguuggca

SEQ ID NO: 19 - DNA, 21 bp, Artificial Sequence
  Chemically modified oligonucleotide
  misc_feature (1)..(21): (1,8,9,10,11,12,13,14,15,16,17,18,19,20,21)=RNA
  misc_feature (2)..(7): (2,3,4,5,6,7)=DNA
uacttggagaaugaguuggca

SEQ ID NO: 20 - RNA, 21 nt, Artificial Sequence
  Positive control sequence
gucaucacacugaauaccaau

SEQ ID NO: 21 - RNA, 23 nt, Artificial Sequence
  Positive control sequence
auugguauucagugugaugacac

SEQ ID NO: 22 - DNA, 32 bp, Artificial Sequence
  Primer sequence
ctagcgagtgccaactcattctccaagtaaat

SEQ ID NO: 23 - DNA, 32 bp, Artificial Sequence
  Primer sequence
ctagatttacttggagaatgagttggcactcg

SEQ ID NO: 24 - RNA, 19 nt, Artificial Sequence
  Chemically modified oligonucleotide
  modified_base (1)..(19): (1,2,18,19)=2'-O-methyl(2'-OMe)
  modified_base (6)..(12): (6,9,10,12)=2'-fluoro
  modified_base (17)..(19): (17,18,19)=phosphorothioate (PS) backbone modification
ccaacucauucuccaaguc

SEQ ID NO: 25 - RNA, 21 nt, Artificial Sequence
  Chemically modified oligonucleotide
  modified_base (1)..(21): (1,3,4,5,12,16,17,20,21)=2'-fluoro
  modified_base (20)..(21): (20,21)=phosphorothioate (PS) backbone modification
uacuuggagaaugaguuggca